European Patent Specification EP 3 972 578 B1, published July 5, 2023. Title: A PHARMACEUTICAL COMPOSITION OF S1PR MODULATORS. Applicant: Università degli Studi di Firenze. The sequence listing filed with the application follows.

SEQUENCE LISTING (5 sequences)

SEQ ID NO: 1 - RNA, 19 nt, Artificial Sequence
  short interfering RNA
cgggguccucugcaaguga

SEQ ID NO: 2 - RNA, 20 nt, Artificial Sequence
  direct primer
gcagccaagaagagaaagaa

SEQ ID NO: 3 - RNA, 19 nt, Artificial Sequence
  forward primer
ctgtgactttgctatcagc

SEQ ID NO: 4 - RNA, 21 nt, Artificial Sequence
  direct primer
ggcaaattcaacggcacagtc

SEQ ID NO: 5 - RNA, 19 nt, Artificial Sequence
  forward primer
tcgctcctggaagatggtg